European Patent Application EP 4 400 508 A1, published July 17, 2024. Title: Active Peptide and Use Thereof. Applicant: HARVEST BIOTECH CO., LTD, Yunnan Botanee Bio-technology Group Co., Ltd. The sequence listing filed with the application follows.

SEQUENCE LISTING (14 sequences)

SEQ ID NO: 1 - protein, 9 aa, Artificial Sequence
  EQ-9
ESETRILLQ

SEQ ID NO: 2 - protein, 9 aa, Artificial Sequence
  EQ-9-1
ESETKILLQ

SEQ ID NO: 3 - protein, 9 aa, Artificial Sequence
  DQ-9
DSDAKILIQ

SEQ ID NO: 4 - protein, 9 aa, Artificial Sequence
  DQ-9-2
DSDAKLLIQ

SEQ ID NO: 5 - protein, 9 aa, Artificial Sequence
  EE-9-1
ETDTRILVE

SEQ ID NO: 6 - protein, 9 aa, Artificial Sequence
  EE-9-2
ESEARIILE

SEQ ID NO: 7 - protein, 9 aa, Artificial Sequence
  DD-9
DSESKLVID

SEQ ID NO: 8 - protein, 9 aa, Artificial Sequence
  EQ-9-2
ESETEAVLQ

SEQ ID NO: 9 - protein, 9 aa, Artificial Sequence
  EQ-9-3
ESKIRILLQ

SEQ ID NO: 10 - protein, 6 aa, Artificial Sequence
  EL-6
ETRILL

SEQ ID NO: 11 - protein, 6 aa, Artificial Sequence
  SL-6
SETRIL

SEQ ID NO: 12 - protein, 17 aa, Artificial Sequence
  LQ-17
LSDQVPDTESETRILLQ

SEQ ID NO: 13 - protein, 13 aa, Artificial Sequence
  VQ-13
VPDTESETRILLQ

SEQ ID NO: 14 - protein, 12 aa, Artificial Sequence
  LT-12
LSDQVPDTESET